European Patent Application EP 4 589 016 A2, published July 23, 2025. Title: GENERATING CAPTURE PROBES FOR SPATIAL ANALYSIS. Applicant: 10x Genomics, Inc. Application EP, filed November 13, 2020. The sequence listing filed with the application follows.

SEQUENCE LISTING (34 sequences)

SEQ ID NO: 1 - protein, 16 aa, synthetic construct
  REGION 1..16: note = Synthetic polypeptide
RADARADARADARADA

SEQ ID NO: 2 - protein, 16 aa, synthetic construct
  REGION 1..16: note = Synthetic EAK16 polypeptide
AEAEAKAKAEAEAKAK

SEQ ID NO: 3 - protein, 12 aa, synthetic construct
  REGION 1..12: note = Synthetic KLD12 polypeptide
KLDLKLDLKLDL

SEQ ID NO: 4 - DNA, 18 bp, synthetic construct
  misc_feature 1..18: note = 18s cDNA Probe 1
  source 1..18: mol_type = other DNA
gaggaattcccagtaagt

SEQ ID NO: 5 - DNA, 18 bp, synthetic construct
  misc_feature 1..18: note = 18S cDNA Probe 2
  source 1..18: mol_type = other DNA
gagattgagcaataacag

SEQ ID NO: 6 - DNA, 18 bp, synthetic construct
  misc_feature 1..18: note = 18s cDNA Probe 3
  source 1..18: mol_type = other DNA
gtagttccgaccataaac

SEQ ID NO: 7 - DNA, 18 bp, synthetic construct
  misc_feature 1..18: note = 18s cDNA Probe 4
  source 1..18: mol_type = other DNA
ggtgactctagataacct

SEQ ID NO: 8 - RNA, 35 nt, synthetic construct
  misc_feature 1..35: note = Analyte poly(A) tail from biological sample
  misc_difference 12..35: note = n is a, c, g, or u
  source 1..35: mol_type = other RNA
aaaaaaaaaaannnnnnnnnnnnnnnnnnnnnnnn

SEQ ID NO: 9 - skipped

SEQ ID NO: 10 - DNA, 18 bp, synthetic construct
  misc_feature 1..18: note = Splint Oligonucleotide
  source 1..18: mol_type = other DNA
aaaaaaaaaacgggccgc

SEQ ID NO: 11 - DNA, 27 bp, synthetic construct
  misc_feature 1..27: note = Capture domain poly(T) sequence
  source 1..27: mol_type = other DNA
ttttttttttttttttttttttttttt

SEQ ID NO: 12 - skipped

SEQ ID NO: 13 - DNA, 14 bp, synthetic construct
  misc_feature 1..14: note = Universal Splint Oligonucleotide
  source 1..14: mol_type = other DNA
tcgactacgtagcg

SEQ ID NO: 14 - skipped

SEQ ID NO: 15 - DNA, 37 bp, synthetic construct
  misc_feature 1..37: note = T30VN
  source 1..37: mol_type = other DNA
tagtcgatttttttttttttttttttttttttttttt

SEQ ID NO: 16-18 - skipped (3 entries)

SEQ ID NO: 19 - DNA, 28 bp, synthetic construct
  misc_feature 1..28: note = Capture Sequence with Ligation Handle
  source 1..28: mol_type = other DNA
tagtcgattgctaggaccggccttaagc

SEQ ID NO: 20 - DNA, 21 bp, synthetic construct
  misc_feature 1..21: note = Capture Sequence Domain of Capture Sequence
  source 1..21: mol_type = other DNA
ttgctaggaccggccttaagc

SEQ ID NO: 21 - DNA, 22 bp, synthetic construct
  misc_feature 1..22: note = Splint Oligonucleotide V2-1
  source 1..22: mol_type = other DNA
gctagtaaggtgcgcaatcctc

SEQ ID NO: 22 - DNA, 22 bp, synthetic construct
  misc_feature 1..22: note = Splint Oligonucleotide V2-2
  source 1..22: mol_type = other DNA
gcaccttggaccgctaaagttg

SEQ ID NO: 23 - DNA, 22 bp, synthetic construct
  misc_feature 1..22: note = Splint Oligonucleotide V2-3
  source 1..22: mol_type = other DNA
gctagtcgagccgacaattgtc

SEQ ID NO: 24 - DNA, 22 bp, synthetic construct
  misc_feature 1..22: note = Splint Oligonucleotide V2-4
  source 1..22: mol_type = other DNA
gcctgacgaaccggttttgcaa

SEQ ID NO: 25 - DNA, 55 bp, synthetic construct
  misc_feature 1..55: note = Donor Oligonucleotide UMI-V2-1
  misc_difference 12..23: note = n is a, c, g, or t
  misc_difference 55: note = n is a, c, g, or t
  source 1..55: mol_type = other DNA
accttactagcnnnnnnnnnnnnttttttttttttttttttttttttttttttvn

SEQ ID NO: 26 - DNA, 55 bp, synthetic construct
  misc_feature 1..55: note = Donor Oligonucleotide UMI-V2-2
  misc_difference 12..23: note = n is a, c, g, or t
  misc_difference 55: note = n is a, c, g, or t
  source 1..55: mol_type = other DNA
gtccaaggtgcnnnnnnnnnnnnttttttttttttttttttttttttttttttvn

SEQ ID NO: 27 - DNA, 55 bp, synthetic construct
  misc_feature 1..55: note = Donor Oligonucleotide UMI-V2-3
  misc_difference 12..23: note = n is a, c, g, or t
  misc_difference 55: note = n is a, c, g, or t
  source 1..55: mol_type = other DNA
gctcgactagcnnnnnnnnnnnnttttttttttttttttttttttttttttttvn

SEQ ID NO: 28 - DNA, 55 bp, synthetic construct
  misc_feature 1..55: note = Donor Oligonucleotide UMI-V2-4
  misc_difference 12..23: note = n is a, c, g, or t
  misc_difference 55: note = n is a, c, g, or t
  source 1..55: mol_type = other DNA
gttcgtcaggcnnnnnnnnnnnnttttttttttttttttttttttttttttttvn

SEQ ID NO: 29 - DNA, 55 bp, synthetic construct; identical to SEQ ID NO: 25
  misc_feature 1..55: note = Donor Oligonucleotide UMI-Cy3
  misc_difference 12..23: note = n is a, c, g, or t
  misc_difference 55: note = n is a, c, g, or t
  source 1..55: mol_type = other DNA

SEQ ID NO: 30 - DNA, 11 bp, synthetic construct
  misc_feature 1..11: note = Acceptor Oligonucleotide Ligation Handle V2-1
  source 1..11: mol_type = other DNA
gaggattgcgc

SEQ ID NO: 31 - DNA, 11 bp, synthetic construct
  misc_feature 1..11: note = Acceptor Oligonucleotide Ligation Handle V2-2
  source 1..11: mol_type = other DNA
caactttagcg

SEQ ID NO: 32 - DNA, 11 bp, synthetic construct
  misc_feature 1..11: note = Acceptor Oligonucleotide Ligation Handle V2-3
  source 1..11: mol_type = other DNA
gacaattgtcg

SEQ ID NO: 33 - skipped

SEQ ID NO: 34 - DNA, 22 bp, synthetic construct
  misc_feature 1..22: note = Blocking Probe
  source 1..22: mol_type = other DNA
agatcggaagagcgtcgtgtag